European Patent Application EP 4 663 183 A1, published December 17, 2025. Title: 재조합 안정화 갈렉틴 9 단백질을 포함하는 안정화된 제제. Applicant: (주)지바이오로직스. Application KR. The sequence listing filed with the application follows.

SEQUENCE LISTING (3 sequences)

SEQ ID NO: 1 - protein, 284 aa, synthetic construct
  REGION 1..284: note = sGal-9
MAFSGSQAPYLSPAVPFSGTIQGGLQDGLQITVNGTVLSSSGTRFAVNFQTGFSGNDIAFHFNPRFEDGGYVVCNTRQNGSWGPEERKTHMPFQKGMPFDLCFLVQSSDFKVMVNGILFVQYFHRVPFHRVDTISVNGSVQLSYISFQHPPYPMPFITTILGGLYPSKSILLSGTVLPSAQRFHINLCSGNHIAFHLNPRFDENAVVRNTQIDNSWGSEERSLPRKMPFVRGQSFSVWILCEAHCLKVAVDGQHLFEYYHRLRNLPTINRLEVGGDIQLTHVQT

SEQ ID NO: 2 - protein, 146 aa, synthetic construct
  REGION 1..146: note = CCRD
TPAIPPMMYPHPAYPMPFITTILGGLYPSKSILLSGTVLPSAQRFHINLCSGNHIAFHLNPRFDENAVVRNTQIDNSWGSEERSLPRKMPFVRGQSFSVWILCEAHCLKVAVDGQHLFEYYHRLRNLPTINRLEVGGDIQLTHVQT

SEQ ID NO: 3 - protein, 10 aa, synthetic construct
  REGION 1..10: note = CCRD 1-10
TPAIPPMMYP